European Patent Application EP 4 241 774 A1, published September 13, 2023. Title: Composition for preventing or treating of neuroinflammatory disease comprising Chlorpromazine. Applicant: OATC Inc Daegu Gyeongbuk Institute of Science and Technology. The sequence listing filed with the application follows.

SEQUENCE LISTING (22 sequences)

SEQ ID NO: 1 - DNA, 1347 bp, Artificial Sequence
  Psen2 N141I
atgctcgcattcatggcctctgacagcgaggaagaggtgtgtgatgagcggacgtccttgatgtcagccgagagccccacatctcgctcctgccaggaaggcaggccaggcccggaggatggagagagcactgcccagtggaggactcaggagagcgaagaagactgtgaagaggacccggaccgctacgcatgcagtggggctcctgggcgaccgtcgggcctggaggaagagctgaccctcaagtatggggcgaagcatgtgatcatgctattcgtgcctgtcacgctgtgtatgatcgtggtggtggccactatcaagtctgtgcgtttctacactgagaagaacgggcagctcatctacacgcccttcacggaggacacgccctcggtgggccagcggctcctcaactccgtgcttatcaccctcatcatgatcagcgtcatcgtagtcatgaccatcttcctcgtggtactctacaagtatcgatgctacaagttcatccatggctggctgatcatgtcctccctgatgctcctcttcttgttcacctacatctacctcggggaagtgctcaagacctacaatgtggccatggactatcccacactcttcctggctgtctggaacttcggggcagtgggcatggtgtgcatccactggaaggggcctctggtgctgcagcaggcttaccttattgtgatcagcgcactcatggccctggtgttcatcaagtacctgccggagtggtctgcctgggtcatcttgggtgccatctctgtgtacgatctcgtggccgtgctgtgccccaaagggccactgaggatgctggtggaaactgcccaggagagaaatgagcccatatttcctgccctgatatactcatctgccatggtgtggacggtgggcatggcaaagctggacccctcctctcaaggagcgctgcagctcccctatgacccagagatggaagaagactcctacgacagttttggagaaccctcataccctgaagccttcgaagcccccctgcctggctacccaggggaggagctggaggaggaggaggaaaggggcgtgaagctcggcctgggagacttcatcttctacagcgtcctggtgggcaaggctgcagccactggcaacggagactggaacactacgctggcctgttttatcgccatcctcattggcttgtgtctcaccctcctgctgcttgctgtgttcaagaaggctctgcccgccctccccatctccatcacctttggactcatcttctacttctccacagacaacctggtgcgccctttcatggacactctggcctcccaccagctctacatctga

SEQ ID NO: 2 - DNA, 1347 bp, Artificial Sequence; identical to SEQ ID NO: 1
  Psen2 wild type

SEQ ID NO: 3 - DNA, 23 bp, Artificial Sequence
  Primer(F) for IL-6
ctggatataatcaggaaatttgc

SEQ ID NO: 4 - DNA, 22 bp, Artificial Sequence
  Primer(R) for IL-6
aaatcttttacctcttggttga

SEQ ID NO: 5 - DNA, 20 bp, Artificial Sequence
  Primer(F) for Cxcl1
catggctgggattcacctca

SEQ ID NO: 6 - DNA, 20 bp, Artificial Sequence
  Primer(R) for Cxcl1
tgaggtgaatcccagccatg

SEQ ID NO: 7 - DNA, 20 bp, Artificial Sequence
  Primer(F) for Ccl2
gtccctgtcatgcttctggg

SEQ ID NO: 8 - DNA, 20 bp, Artificial Sequence
  Primer(R) for Ccl2
ccccaagaaggaatgggtcc

SEQ ID NO: 9 - DNA, 20 bp, Artificial Sequence
  Primer(F) for Ccl5
cctcaccatatggctcggac

SEQ ID NO: 10 - DNA, 20 bp, Artificial Sequence
  Primer(R) for Ccl5
tgctccaatcttgcagtcgt

SEQ ID NO: 11 - DNA, 25 bp, Artificial Sequence
  Primer(F) for Tnf
catcttctcaaaattcgagtgacaa

SEQ ID NO: 12 - DNA, 23 bp, Artificial Sequence
  Primer(R) for Tnf
tgggagtagacaaggtacaaccc

SEQ ID NO: 13 - DNA, 20 bp, Artificial Sequence
  Primer(F) for Actb
agagggaaatcgtgcgtgac

SEQ ID NO: 14 - DNA, 21 bp, Artificial Sequence
  Primer(R) for Actb
caatagtgatgacctggccgt

SEQ ID NO: 15 - DNA, 18 bp, Artificial Sequence
  Primer(F) for Il-1b
aggccacaggtattttgt

SEQ ID NO: 16 - DNA, 18 bp, Artificial Sequence
  Primer(R) for Il-1b
gcccatcctctgtgactc

SEQ ID NO: 17 - DNA, 20 bp, Artificial Sequence
  Primer(F) for Actb
agagggaaatcgtgcgtgac

SEQ ID NO: 18 - DNA, 21 bp, Artificial Sequence
  Primer(R) for Actb
caatagtgatgacctggccgt

SEQ ID NO: 19 - DNA, 20 bp, Artificial Sequence
  Primer(F) for Nr1d1
tgctggcatgtcccatgaac

SEQ ID NO: 20 - DNA, 20 bp, Artificial Sequence
  Primer(R) for Nr1d1
gactgtaggttgtgcggctc

SEQ ID NO: 21 - DNA, 20 bp, Artificial Sequence
  Primer(F) for Actb
agagggaaatcgtgcgtgac

SEQ ID NO: 22 - DNA, 21 bp, Artificial Sequence
  Primer(R) for Actb
caatagtgatgacctggccgt